European Patent Application EP 4 230 738 A1, published August 23, 2023. Title: Prime editing-based gene editing composition with improved editing efficiency and use thereof. Applicant: Korea University Research and Business Foundation Seoul National University R&DB Foundation Korea Mouse Phenotyping Center. The sequence listing filed with the application follows.

SEQUENCE LISTING (73 sequences)

SEQ ID NO: 1 - protein, 2308 aa, Artificial Sequence
  CMP-PE-V1
MKRTADGSEFESPKKKRKVMPKRKVSSAEGAAKEEPKRRSARLSAKPPAKVEAKPKKAAAKDKSSDKKVQTKGKRGAKGKQAEVANQETKEDLPAENGETKTEESPASDEAGEKEAKSDTGSGDKKYSIGLDIGTNSVGWAVITDEYKVPSKKFKVLGNTDRHSIKKNLIGALLFDSGETAEATRLKRTARRRYTRRKNRICYLQEIFSNEMAKVDDSFFHRLEESFLVEEDKKHERHPIFGNIVDEVAYHEKYPTIYHLRKKLVDSTDKADLRLIYLALAHMIKFRGHFLIEGDLNPDNSDVDKLFIQLVQTYNQLFEENPINASGVDAKAILSARLSKSRRLENLIAQLPGEKKNGLFGNLIALSLGLTPNFKSNFDLAEDAKLQLSKDTYDDDLDNLLAQIGDQYADLFLAAKNLSDAILLSDILRVNTEITKAPLSASMIKRYDEHHQDLTLLKALVRQQLPEKYKEIFFDQSKNGYAGYIDGGASQEEFYKFIKPILEKMDGTEELLVKLNREDLLRKQRTFDNGSIPHQIHLGELHAILRRQEDFYPFLKDNREKIEKILTFRIPYYVGPLARGNSRFAWMTRKSEETITPWNFEEVVDKGASAQSFIERMTNFDKNLPNEKVLPKHSLLYEYFTVYNELTKVKYVTEGMRKPAFLSGEQKKAIVDLLFKTNRKVTVKQLKEDYFKKIECFDSVEISGVEDRFNASLGTYHDLLKIIKDKDFLDNEENEDILEDIVLTLTLFEDREMIEERLKTYAHLFDDKVMKQLKRRRYTGWGRLSRKLINGIRDKQSGKTILDFLKSDGFANRNFMQLIHDDSLTFKEDIQKAQVSGQGDSLHEHIANLAGSPAIKKGILQTVKVVDELVKVMGRHKPENIVIEMARENQTTQKGQKNSRERMKRIEEGIKELGSQILKEHPVENTQLQNEKLYLYYLQNGRDMYVDQELDINRLSDYDVDAIVPQSFLKDDSIDNKVLTRSDKNRGKSDNVPSEEVVKKMKNYWRQLLNAKLITQRKFDNLTKAERGGLSELDKAGFIKRQLVETRQITKHVAQILDSRMNTKYDENDKLIREVKVITLKSKLVSDFRKDFQFYKVREINNYHHAHDAYLNAVVGTALIKKYPKLESEFVYGDYKVYDVRKMIAKSEQEIGKATAKYFFYSNIMNFFKTEITLANGEIRKRPLIETNGETGEIVWDKGRDFATVRKVLSMPQVNIVKKTEVQTGGFSKESILPKRNSDKLIARKKDWDPKKYGGFDSPTVAYSVLVVAKVEKGKSKKLKSVKELLGITIMERSSFEKNPIDFLEAKGYKEVKKDLIIKLPKYSLFELENGRKRMLASAGELQKGNELALPSKYVNFLYLASHYEKLKGSPEDNEQKQLFVEQHKHYLDEIIEQISEFSKRVILADANLDKVLSAYNKHRDKPIREQAENIIHLFTLTNLGAPAAFKYFDTTIDRKRYTSTKEVLDATLIHQSITGLYETRIDLSQLGGDLEGGGGSSTDHPKYSDMIVAAIQAEKNRAGSSRQSIQKYIKSHYKVGENADSQIKLSIKRLVTTGVLKQTKGVGASGSFRLAKSDEPSGGSSGGSSGSETPGTSESATPESSGGSSGGSSTLNIEDEYRLHETSKEPDVSLGSTWLSDFPQAWAETGGMGLAVRQAPLIIPLKATSTPVSIKQYPMSQEARLGIKPHIQRLLDQGILVPCQSPWNTPLLPVKKPGTNDYRPVQDLREVNKRVEDIHPTVPNPYNLLSGLPPSHQWYTVLDLKDAFFCLRLHPTSQPLFAFEWRDPEMGISGQLTWTRLPQGFKNSPTLFNEALHRDLADFRIQHPDLILLQYVDDLLLAATSELDCQQGTRALLQTLGNLGYRASAKKAQICQKQVKYLGYLLKEGQRWLTEARKETVMGQPTPKTPRQLREFLGKAGFCRLFIPGFAEMAAPLYPLTKPGTLFNWGPDQQKAYQEIKQALLTAPALGLPDLTKPFELFVDEKQGYAKGVLTQKLGPWRRPVAYLSKKLDPVAAGWPPCLRMVAAIAVLTKDAGKLTMGQPLVILAPHAVEALVKQPPDRWLSNARMTHYQALLLDTDRVQFGPVVALNPATLLPLPEEGLQHNCLDILAEAHGTRPDLTDQPLPDADHTWYTDGSSLLQEGQRKAGAAVTTETEVIWAKALPAGTSAQRAELIALTQALKMAEGKKLNVYTDSRYAFATAHIHGEIYRRRGWLTSEGKEIKNKDEILALLKALFLPKRLSIIHCPGHQKGHSAEARGNRMADQAARKAAITETPDTSTLLIENSSPSGGSKRTADGSEFEPKKKRKV

SEQ ID NO: 2 - protein, 2308 aa, Artificial Sequence
  CMP-PE-V2
MKRTADGSEFESPKKKRKVMPKRKVSSAEGAAKEEPKRRSARLSAKPPAKVEAKPKKAAAKDKSSDKKVQTKGKRGAKGKQAEVANQETKEDLPAENGETKTEESPASDEAGEKEAKSDTGSGDKKYSIGLDIGTNSVGWAVITDEYKVPSKKFKVLGNTDRHSIKKNLIGALLFDSGETAEATRLKRTARRRYTRRKNRICYLQEIFSNEMAKVDDSFFHRLEESFLVEEDKKHERHPIFGNIVDEVAYHEKYPTIYHLRKKLVDSTDKADLRLIYLALAHMIKFRGHFLIEGDLNPDNSDVDKLFIQLVQTYNQLFEENPINASGVDAKAILSARLSKSRRLENLIAQLPGEKKNGLFGNLIALSLGLTPNFKSNFDLAEDAKLQLSKDTYDDDLDNLLAQIGDQYADLFLAAKNLSDAILLSDILRVNTEITKAPLSASMIKRYDEHHQDLTLLKALVRQQLPEKYKEIFFDQSKNGYAGYIDGGASQEEFYKFIKPILEKMDGTEELLVKLNREDLLRKQRTFDNGSIPHQIHLGELHAILRRQEDFYPFLKDNREKIEKILTFRIPYYVGPLARGNSRFAWMTRKSEETITPWNFEEVVDKGASAQSFIERMTNFDKNLPNEKVLPKHSLLYEYFTVYNELTKVKYVTEGMRKPAFLSGEQKKAIVDLLFKTNRKVTVKQLKEDYFKKIECFDSVEISGVEDRFNASLGTYHDLLKIIKDKDFLDNEENEDILEDIVLTLTLFEDREMIEERLKTYAHLFDDKVMKQLKRRRYTGWGRLSRKLINGIRDKQSGKTILDFLKSDGFANRNFMQLIHDDSLTFKEDIQKAQVSGQGDSLHEHIANLAGSPAIKKGILQTVKVVDELVKVMGRHKPENIVIEMARENQTTQKGQKNSRERMKRIEEGIKELGSQILKEHPVENTQLQNEKLYLYYLQNGRDMYVDQELDINRLSDYDVDAIVPQSFLKDDSIDNKVLTRSDKNRGKSDNVPSEEVVKKMKNYWRQLLNAKLITQRKFDNLTKAERGGLSELDKAGFIKRQLVETRQITKHVAQILDSRMNTKYDENDKLIREVKVITLKSKLVSDFRKDFQFYKVREINNYHHAHDAYLNAVVGTALIKKYPKLESEFVYGDYKVYDVRKMIAKSEQEIGKATAKYFFYSNIMNFFKTEITLANGEIRKRPLIETNGETGEIVWDKGRDFATVRKVLSMPQVNIVKKTEVQTGGFSKESILPKRNSDKLIARKKDWDPKKYGGFDSPTVAYSVLVVAKVEKGKSKKLKSVKELLGITIMERSSFEKNPIDFLEAKGYKEVKKDLIIKLPKYSLFELENGRKRMLASAGELQKGNELALPSKYVNFLYLASHYEKLKGSPEDNEQKQLFVEQHKHYLDEIIEQISEFSKRVILADANLDKVLSAYNKHRDKPIREQAENIIHLFTLTNLGAPAAFKYFDTTIDRKRYTSTKEVLDATLIHQSITGLYETRIDLSQLGGDSGGSSGGSSGSETPGTSESATPESSGGSSGGSSTLNIEDEYRLHETSKEPDVSLGSTWLSDFPQAWAETGGMGLAVRQAPLIIPLKATSTPVSIKQYPMSQEARLGIKPHIQRLLDQGILVPCQSPWNTPLLPVKKPGTNDYRPVQDLREVNKRVEDIHPTVPNPYNLLSGLPPSHQWYTVLDLKDAFFCLRLHPTSQPLFAFEWRDPEMGISGQLTWTRLPQGFKNSPTLFNEALHRDLADFRIQHPDLILLQYVDDLLLAATSELDCQQGTRALLQTLGNLGYRASAKKAQICQKQVKYLGYLLKEGQRWLTEARKETVMGQPTPKTPRQLREFLGKAGFCRLFIPGFAEMAAPLYPLTKPGTLFNWGPDQQKAYQEIKQALLTAPALGLPDLTKPFELFVDEKQGYAKGVLTQKLGPWRRPVAYLSKKLDPVAAGWPPCLRMVAAIAVLTKDAGKLTMGQPLVILAPHAVEALVKQPPDRWLSNARMTHYQALLLDTDRVQFGPVVALNPATLLPLPEEGLQHNCLDILAEAHGTRPDLTDQPLPDADHTWYTDGSSLLQEGQRKAGAAVTTETEVIWAKALPAGTSAQRAELIALTQALKMAEGKKLNVYTDSRYAFATAHIHGEIYRRRGWLTSEGKEIKNKDEILALLKALFLPKRLSIIHCPGHQKGHSAEARGNRMADQAARKAAITETPDTSTLLIENSSPSGGSLEGGGGSSTDHPKYSDMIVAAIQAEKNRAGSSRQSIQKYIKSHYKVGENADSQIKLSIKRLVTTGVLKQTKGVGASGSFRLAKSDEPKRTADGSEFEPKKKRKV

SEQ ID NO: 3 - DNA, 20 bp, Artificial Sequence
  tdTomato_G to C / T ins_8-17_spacer
cgcatggagggctccatgaa

SEQ ID NO: 4 - DNA, 8 bp, Artificial Sequence
  tdTomato_G to C / T ins_8-17_PBS
atggagcc

SEQ ID NO: 5 - DNA, 17 bp, Artificial Sequence
  tdTomato_G to C / T ins_8-17_RT template
gaactcagtggcggttc

SEQ ID NO: 6 - DNA, 20 bp, Artificial Sequence
  Igf2_G to C / TA ins_9-14_Spacer
tattggaagaacttgcccac

SEQ ID NO: 7 - DNA, 9 bp, Artificial Sequence
  Igf2_G to C / TA ins_9-14_PBS
ggcaagttc

SEQ ID NO: 8 - DNA, 14 bp, Artificial Sequence
  Igf2_G to C / TA ins_9-14_RT template
agataccgcgtgta

SEQ ID NO: 9 - DNA, 20 bp, Artificial Sequence
  Adamts20_CG to AA_11-13_Spacer
agtgaataagaagacgtact

SEQ ID NO: 10 - DNA, 11 bp, Artificial Sequence
  Adamts20_CG to AA_11-13_PBS
acgtcttctta

SEQ ID NO: 11 - DNA, 13 bp, Artificial Sequence
  Adamts20_CG to AA_11-13_RT template
gaccggccttagt

SEQ ID NO: 12 - DNA, 20 bp, Artificial Sequence
  Casp1_TAGG del_12-12_Spacer
gtcttgtctcttataggaga

SEQ ID NO: 13 - DNA, 12 bp, Artificial Sequence
  Casp1_TAGG del_12-12_PBS
cctataagagac

SEQ ID NO: 14 - DNA, 12 bp, Artificial Sequence
  Casp1_TAGG del_12-12_RT template
acctctttcact

SEQ ID NO: 15 - DNA, 20 bp, Artificial Sequence
  Hoxd13_G to T_10-15_Spacer
gaggcatacatctccatgga

SEQ ID NO: 16 - DNA, 10 bp, Artificial Sequence
  Hoxd13_G to T_10-15_PBS
atggagatgt

SEQ ID NO: 17 - DNA, 15 bp, Artificial Sequence
  Hoxd13_G to T_10-15_RT template
gactggtagacctcc

SEQ ID NO: 18 - DNA, 20 bp, Artificial Sequence
  Angpt1_CGG to TGA_11-13_Spacer
cacattgcccatgttgaatc

SEQ ID NO: 19 - DNA, 11 bp, Artificial Sequence
  Angpt1_CGG to TGA_11-13_PBS
tcaacatgggc

SEQ ID NO: 20 - DNA, 13 bp, Artificial Sequence
  Angpt1_CGG to TGA_11-13_RT template
gatataactgaat

SEQ ID NO: 21 - DNA, 20 bp, Artificial Sequence
  Ksr2_TGAT ins_8-14_Spacer
tcctgccctggctccgtggt

SEQ ID NO: 22 - DNA, 8 bp, Artificial Sequence
  Ksr2_TGAT ins_8-14_PBS
acggagcc

SEQ ID NO: 23 - DNA, 14 bp, Artificial Sequence
  Ksr2_TGAT ins_8-14_RT template
gtggcccacctgat

SEQ ID NO: 24 - DNA, 20 bp, Artificial Sequence
  Ar_G to T_13-13_Spacer
tctcacttgtggcagctgca

SEQ ID NO: 25 - DNA, 13 bp, Artificial Sequence
  Ar_G to T_13-13_PBS
agctgccacaagt

SEQ ID NO: 26 - DNA, 13 bp, Artificial Sequence
  Ar_G to T_13-13_RT template
aagaagaccttga

SEQ ID NO: 27 - DNA, 20 bp, Artificial Sequence
  tdTomato-nsgRNA
gccctcgatctcgaactcag

SEQ ID NO: 28 - DNA, 20 bp, Artificial Sequence
  Igf2-nsgRNA
cttccccagataccgcgtgt

SEQ ID NO: 29 - DNA, 20 bp, Artificial Sequence
  Adamt20-nsgRNA
agctcgtgttcaaggacatg

SEQ ID NO: 30 - DNA, 20 bp, Artificial Sequence
  Casp1-nsgRNA
ctgtcagaagtcttgtgctc

SEQ ID NO: 31 - DNA, 20 bp, Artificial Sequence
  Hoxd13-nsgRNA
gatccttggcacagtacacc

SEQ ID NO: 32 - DNA, 20 bp, Artificial Sequence
  Angpt1-nsgRNA
gatataactgaattcaacat

SEQ ID NO: 33 - DNA, 20 bp, Artificial Sequence
  Ksr2-nsgRNA
acctgatacggagccagggc

SEQ ID NO: 34 - DNA, 20 bp, Artificial Sequence
  Ar-nsgRNA
aggggaaaatatcaggaagt

SEQ ID NO: 35 - DNA, 14 bp, Artificial Sequence
  Igf2_dsgRNA_-34
agtcagcaggtttc

SEQ ID NO: 36 - DNA, 14 bp, Artificial Sequence
  Igf2_dsgRNA_-27
aggtgctagtcagc

SEQ ID NO: 37 - DNA, 14 bp, Artificial Sequence
  Igf2_dsgRNA_+7
tggagacagtccgc

SEQ ID NO: 38 - DNA, 14 bp, Artificial Sequence
  Igf2_dsgRNA_+22
ggacgcctgcgcag

SEQ ID NO: 39 - DNA, 14 bp, Artificial Sequence
  Adamts20_dsgRNA_-13
tcaagagcacagcc

SEQ ID NO: 40 - DNA, 14 bp, Artificial Sequence
  Adamts20_dsgRNA_+14
tttctggtgcttgg

SEQ ID NO: 41 - DNA, 14 bp, Artificial Sequence
  Adamts20_dsgRNA_+24
cgattttgactttc

SEQ ID NO: 42 - DNA, 14 bp, Artificial Sequence
  Adamts20_dsgRNA_+41
cttccgctcacttc

SEQ ID NO: 43 - DNA, 14 bp, Artificial Sequence
  Casp1_dsgRNA_-13
ctttgacttctcta

SEQ ID NO: 44 - DNA, 15 bp, Artificial Sequence
  Casp1_dsgRNA_-12
actttgacttctcta

SEQ ID NO: 45 - DNA, 14 bp, Artificial Sequence
  Casp1_dsgRNA_+7
cagcaaattctttc

SEQ ID NO: 46 - DNA, 14 bp, Artificial Sequence
  Casp1_dsgRNA_+62
gtattcatgtctca

SEQ ID NO: 47 - DNA, 14 bp, Artificial Sequence
  Hoxd13_dsgRNA_-12
cccggatccaaaag

SEQ ID NO: 48 - DNA, 14 bp, Artificial Sequence
  Hoxd13_dsgRNA_-11
cacttttggatccg

SEQ ID NO: 49 - DNA, 14 bp, Artificial Sequence
  Hoxd13_dsgRNA_+20
gctgttccacccgt

SEQ ID NO: 50 - DNA, 14 bp, Artificial Sequence
  Hoxd13_dsgRNA_+24
cgggtggaacagcc

SEQ ID NO: 51 - DNA, 14 bp, Artificial Sequence
  Angpt1_dsgRNA_-15
cgaaatccagaaaa

SEQ ID NO: 52 - DNA, 14 bp, Artificial Sequence
  Angpt1_dsgRNA_-11
atccagaaaacgga

SEQ ID NO: 53 - DNA, 14 bp, Artificial Sequence
  Angpt1_dsgRNA_+14
cttccagaacacga

SEQ ID NO: 54 - DNA, 14 bp, Artificial Sequence
  Angpt1_dsgRNA_+17
ttcccgtcgtgttc

SEQ ID NO: 55 - DNA, 14 bp, Artificial Sequence
  Ksr2_dsgRNA_-12
tctccaaacaagat

SEQ ID NO: 56 - DNA, 14 bp, Artificial Sequence
  Ksr2_dsgRNA_+7
tccggggggcacac

SEQ ID NO: 57 - DNA, 14 bp, Artificial Sequence
  Ar_dsgRNA_-15
ggagatgaagcttc

SEQ ID NO: 58 - DNA, 27 bp, Artificial Sequence
  Closed chromatin_Forward
gcagcagatggcaagtaatactaagat

SEQ ID NO: 59 - DNA, 30 bp, Artificial Sequence
  Closed chromatin_Reverse
cccttattctctgagcattagacagttata

SEQ ID NO: 60 - DNA, 28 bp, Artificial Sequence
  Open chromatin_Forward
tgagtcacagcatcagcatcgggtctct

SEQ ID NO: 61 - DNA, 28 bp, Artificial Sequence
  Open chromatin_Reverse
ggagagggcctttttctcttcaaggttc

SEQ ID NO: 62 - DNA, 22 bp, Artificial Sequence
  Igf2_Forward
tctccaggacgacttccccaga

SEQ ID NO: 63 - DNA, 24 bp, Artificial Sequence
  Igf2_Reverse
ctccaggtgtcatattggaagaac

SEQ ID NO: 64 - DNA, 19 bp, Artificial Sequence
  Adamts20_Forward
gtggaatcaagagcacagc

SEQ ID NO: 65 - DNA, 20 bp, Artificial Sequence
  Adamts20_Reverse
cagtgaataagaagacgtac

SEQ ID NO: 66 - DNA, 25 bp, Artificial Sequence
  Casp1_Forward
aaatcactggtcttgtctcttatag

SEQ ID NO: 67 - DNA, 23 bp, Artificial Sequence
  Casp1_Reverse
cagcaaattctttcacctctttc

SEQ ID NO: 68 - DNA, 25 bp, Artificial Sequence
  Hoxd13_Forward
tcggcacgaggcatacatctccatg

SEQ ID NO: 69 - DNA, 22 bp, Artificial Sequence
  Hoxd13_Reverse
cgttggctagcgtccaggactg

SEQ ID NO: 70 - DNA, 21 bp, Artificial Sequence
  Angpt1_Forward
ccagaaaacggagggagaaga

SEQ ID NO: 71 - DNA, 21 bp, Artificial Sequence
  Angpt1_Reverse
taggcacattgcccatgttga

SEQ ID NO: 72 - DNA, 24 bp, Artificial Sequence
  Ksr2_Forward
tctctccaaacaagattggatcat

SEQ ID NO: 73 - DNA, 17 bp, Artificial Sequence
  Ksr2_Reverse
tctcctgccctggctcc